European Patent Application EP 4 293 043 A1, published December 20, 2023. Title: EPITOPE PEPTIDE OF RAS G13D MUTANT AND T CELL RECEPTOR RECOGNIZING RAS G13D MUTANT. Applicant: SHANGHAI GENBASE BIOTECHNOLOGY CO., LTD. Application PCT/CN2022/075005. The sequence listing filed with the application follows.

SEQUENCE LISTING (100 sequences)

SEQ ID NO: 1 - DNA, 2012 bp, Artificial Sequence
  Nucleotide sequence of RAS G13D-mRNA
cttgttctttttgcagaagctcagaataaacgctcaactttgggccaccatgccccggcagctcagcgcggcggccgcgctcttcgcgtccctggccgtaattttgcacgatggcagtcaaatgagagcaaaagcatttccagaaaccagagattattctcaacctactgcagcagcaacagtacaggacataaaaaaacctgtccagcaaccagctaagcaagcacctcaccaaactttagcagcaagattcatggatggtcatatcacctttcaaacagcggccacagtaaaaattccaacaactaccccagcgactacaaaaaacactgcaaccaccagcccaattacctacaccctggtcacaacccaggccacacccaacaactcacacacagctcctccagttactgaagttacagtcggccctagcttagccccttattcactgccacccaccatcaccccaccagctcatacaactggaaccagttcatcaaccgtcagccacacaactgggaacaccactcaacccagtaaccagaccacccttccagcaactttatcgatagcactgcacaaaagcacaaccggtcagaagcctgttcaacccacccatgccccaggaacaacggcagctgcccacaataccacccgcacagctgcacctgcctccacggttcctgggcccacccttgcacctcagccatcgtcagtcaagactggaatttatcaggttctaaacggaagcagactctgtataaaagcagagatggggatacagctgattgttcaagacaaggagtcggttttttcacctcggagatacttcaacatcgaccccaacgcaacgcaagcctctgggaactgtggcacccgaaaatccaaccttctgttgaattttcagggcggatttgtgaatctcacatttaccaaggatgaagaatcatattatatcagtgaagtgggagcctatttgaccgtctcagatccagagacaatttaccaaggaatcaaacatgcggtggtgatgttccagacagcagtcgggcattccttcaagtgcgtgagtgaacagagcctccagttgtcagcccacctgcaggtgaaaacaaccgatgtccaacttcaagcctttgattttgaagatgaccactttggaaatgtggatgagtgctcgtctgactacacaactgaatataaacttgtggtagttggagctggcgatgtaggcaagagtgccttgacgatacagctaattcagaatcattttgtggacgaatatgatccaacaatagaggattcctacaggaagcaagtagtaattgatggagaaacctgtctcttggatattctcgacacagcaggtcaagaggagtacagtgcaatgagggaccagtacatgaggactggggagggctttctttgtgtatttgccataaataatactaaatcatttgaagatattcaccattatagagaacaaattaaaagagttaaggactctgaagatgtacctatggtcctagtaggaaataaatgtgatttgccttctagaacagtagacacaaaacaggctcaggacttagcaagaagttatggaattccttttattgaaacatcagcaaagacaagacagggtgttgatgatgccttctatacattagttcgagaaattcgaaaacataaagaaaagatgagcaaagatggtaaaaagaagaaaaagaagtcaaagacaaagtgtgtaattatgattgtgcttcctgtgattggggccatcgtggttggtctctgccttatgggtatgggtgtctataaaatccgcctaaggtgtcaatcatctggataccagagaatctaatcctctagaggatctggttaccactaaaccagcctcaagaacacccgaatggagtctctaagctacataataccaacttacacttacaaaatgttgtcccccaaaatgtagccattcgtatctgctcctaataaaaagaaagtttcttcac

SEQ ID NO: 2 - DNA, 408 bp, Artificial Sequence
  Nucleotide sequence of TCR Valpha
atgtcactttctagcctgctgaaggtggtcacagcttcactgtggctaggacctggcattgcccagaagataactcaaacccaaccaggaatgttcgtgcaggaaaaggaggctgtgactctggactgcacatatgacaccagtgatccaagttatggtctattctggtacaagcagcccagcagtggggaaatgatttttcttatttatcaggggtcttatgaccagcaaaatgcaacagaaggtcgctactcattgaatttccagaaggcaagaaaatccgccaaccttgtcatctccgcttcacaactgggggactcagcaatgtacttctgtgcaatgagagagaggaccggcactgccagtaaactcacctttgggactggaacaagacttcaggtcacgctc

SEQ ID NO: 3 - DNA, 390 bp, Artificial Sequence
  Nucleotide sequence of TCR Vbeta
atgggaatcaggctcctctgtcgtgtggccttttgtttcctggctgtaggcctcgtagatgtgaaagtaacccagagctcgagatatctagtcaaaaggacgggagagaaagtttttctggaatgtgtccaggatatggaccatgaaaatatgttctggtatcgacaagacccaggtctggggctacggctgatctatttctcatatgatgttaaaatgaaagaaaaaggagatattcctgaggggtacagtgtctctagagagaagaaggagcgcttctccctgattctggagtccgccagcaccaaccagacatctatgtacctctgtgccagcagccagacggtgccgccccagcattttggtgatgggactcgactctccatccta

SEQ ID NO: 4 - protein, 136 aa, Artificial Sequence
  Amino acid sequence of TCR Valpha
MSLSSLLKVVTASLWLGPGIAQKITQTQPGMFVQEKEAVTLDCTYDTSDPSYGLFWYKQPSSGEMIFLIYQGSYDQQNATEGRYSLNFQKARKSANLVISASQLGDSAMYFCAMRERTGTASKLTFGTGTRLQVTL

SEQ ID NO: 5 - protein, 130 aa, Artificial Sequence
  Amino acid sequence of TCR Vbeta
MGIRLLCRVAFCFLAVGLVDVKVTQSSRYLVKRTGEKVFLECVQDMDHENMFWYRQDPGLGLRLIYFSYDVKMKEKGDIPEGYSVSREKKERFSLILESASTNQTSMYLCASSQTVPPQHFGDGTRLSIL

SEQ ID NO: 6 - protein, 7 aa, Artificial Sequence
  Amino acid sequence of TCR CDR1alpha
TSDPSYG

SEQ ID NO: 7 - protein, 8 aa, Artificial Sequence
  Amino acid sequence of TCR CDR2alpha
QGSYDQQN

SEQ ID NO: 8 - protein, 13 aa, Artificial Sequence
  Amino acid sequence of TCR CDR3alpha
AMRERTGTASKLT

SEQ ID NO: 9 - protein, 5 aa, Artificial Sequence
  Amino acid sequence of TCR CDR1beta
MDHEN

SEQ ID NO: 10 - protein, 6 aa, Artificial Sequence
  Amino acid sequence of TCR CDR2beta
SYDVKM

SEQ ID NO: 11 - protein, 10 aa, Artificial Sequence
  Amino acid sequence of TCR CDR3beta
ASSQTVPPQH

SEQ ID NO: 12 - protein, 23 aa, Artificial Sequence
  Amino acid sequence of RAS WT23mer
TEYKLVVVGAGGVGKSALTIQLI

SEQ ID NO: 13 - protein, 23 aa, Artificial Sequence
  Amino acid sequence of G13D 23mer
TEYKLVVVGAGDVGKSALTIQLI

SEQ ID NO: 14 - protein, 11 aa, Artificial Sequence
  Epitope peptide core amino acid sequence
VVVGAGDVGKS

SEQ ID NO: 15 - protein, 19 aa, Artificial Sequence
  Amino acid sequence of G13D-RT1
KLVVVGAGDVGKSALTIQL

SEQ ID NO: 16 - protein, 18 aa, Artificial Sequence
  Amino acid sequence of G13D-RT2
KLVVVGAGDVGKSALTIQ

SEQ ID NO: 17 - protein, 17 aa, Artificial Sequence
  Amino acid sequence of G13D-RT3
KLVVVGAGDVGKSALTI

SEQ ID NO: 18 - protein, 17 aa, Artificial Sequence
  Amino acid sequence of G13D-RT4
YKLVVVGAGDVGKSALT

SEQ ID NO: 19 - protein, 16 aa, Artificial Sequence
  Amino acid sequence of G13D-RT5
KLVVVGAGDVGKSALT

SEQ ID NO: 20 - protein, 16 aa, Artificial Sequence
  Amino acid sequence of G13D-RT6
YKLVVVGAGDVGKSAL

SEQ ID NO: 21 - protein, 15 aa, Artificial Sequence
  Amino acid sequence of G13D-RT7
KLVVVGAGDVGKSAL

SEQ ID NO: 22 - protein, 14 aa, Artificial Sequence
  Amino acid sequence of G13D-RT8
LVVVGAGDVGKSAL

SEQ ID NO: 23 - protein, 13 aa, Artificial Sequence
  Amino acid sequence of G13D-RT9
VVVGAGDVGKSAL

SEQ ID NO: 24 - protein, 12 aa, Artificial Sequence
  Amino acid sequence of G13D-RT10
VVGAGDVGKSAL

SEQ ID NO: 25 - protein, 11 aa, Artificial Sequence
  Amino acid sequence of G13D-RT11
VGAGDVGKSAL

SEQ ID NO: 26 - protein, 14 aa, Artificial Sequence
  Amino acid sequence of G13D-RT12
KLVVVGAGDVGKSA

SEQ ID NO: 27 - protein, 13 aa, Artificial Sequence
  Amino acid sequence of G13D-RT13
KLVVVGAGDVGKS

SEQ ID NO: 28 - protein, 12 aa, Artificial Sequence
  Amino acid sequence of G13D-RT14
KLVVVGAGDVGK

SEQ ID NO: 29 - protein, 11 aa, Artificial Sequence
  Amino acid sequence of G13D-RT15
KLVVVGAGDVG

SEQ ID NO: 30 - protein, 16 aa, Artificial Sequence
  Amino acid sequence of G13D-RT6-A1
AKLVVVGAGDVGKSAL

SEQ ID NO: 31 - protein, 16 aa, Artificial Sequence
  Amino acid sequence of G13D-RT6-A2
YALVVVGAGDVGKSAL

SEQ ID NO: 32 - protein, 16 aa, Artificial Sequence
  Amino acid sequence of G13D-RT6-A3
YKAVVVGAGDVGKSAL

SEQ ID NO: 33 - protein, 16 aa, Artificial Sequence
  Amino acid sequence of G13D-RT6-A4
YKLAVVGAGDVGKSAL

SEQ ID NO: 34 - protein, 16 aa, Artificial Sequence
  Amino acid sequence of G13D-RT6-A5
YKLVAVGAGDVGKSAL

SEQ ID NO: 35 - protein, 16 aa, Artificial Sequence
  Amino acid sequence of G13D-RT6-A6
YKLVVAGAGDVGKSAL

SEQ ID NO: 36 - protein, 16 aa, Artificial Sequence
  Amino acid sequence of G13D-RT6-A7
YKLVVVAAGDVGKSAL

SEQ ID NO: 37 - protein, 16 aa, Artificial Sequence
  Amino acid sequence of G13D-RT6-G8
YKLVVVGGGDVGKSAL

SEQ ID NO: 38 - protein, 16 aa, Artificial Sequence
  Amino acid sequence of G13D-RT6-A9
YKLVVVGAADVGKSAL

SEQ ID NO: 39 - protein, 16 aa, Artificial Sequence
  Amino acid sequence of G13D-RT6-A11
YKLVVVGAGDAGKSAL

SEQ ID NO: 40 - protein, 16 aa, Artificial Sequence
  Amino acid sequence of G13D-RT6-A12
YKLVVVGAGDVAKSAL

SEQ ID NO: 41 - protein, 16 aa, Artificial Sequence
  Amino acid sequence of G13D-RT6-A13
YKLVVVGAGDVGASAL

SEQ ID NO: 42 - protein, 16 aa, Artificial Sequence
  Amino acid sequence of G13D-RT6-A14
YKLVVVGAGDVGKAAL

SEQ ID NO: 43 - protein, 16 aa, Artificial Sequence
  Amino acid sequence of G13D-RT6-G15
YKLVVVGAGDVGKSGL

SEQ ID NO: 44 - protein, 16 aa, Artificial Sequence
  Amino acid sequence of G13D-RT6-A16
YKLVVVGAGDVGKSAA

SEQ ID NO: 45 - protein, 137 aa, Artificial Sequence
  Amino acid sequence of murine TCRalpha constant region
DIQNPEPAVYQLKDPRSQDSTLCLFTDFDSQINVPKTMESGTFITDKTVLDMKAMDSKSNGAIAWSNQTSFTCQDIFKETNATYPSSDVPCDATLTEKSFETDMNLNFQNLSVMGLRILLLKVAGFNLLMTLRLWSS

SEQ ID NO: 46 - DNA, 411 bp, Artificial Sequence
  Nucleotide sequence of murine TCRalpha constant region
gacatccagaacccagaacctgctgtgtaccagttaaaagatcctcggtctcaggacagcaccctctgcctgttcaccgactttgactcccaaatcaatgtgccgaaaaccatggaatctggaacgttcatcactgacaaaactgtgctggacatgaaagctatggattccaagagcaatggggccattgcctggagcaaccagacaagcttcacctgccaagatatcttcaaagagaccaacgccacctaccccagttcagacgttccctgtgatgccacgttgactgagaaaagctttgaaacagatatgaacctaaactttcaaaacctgtcagttatgggactccgaatcctcctgctgaaagtagccggatttaacctgctcatgacgctgaggctgtggtccagt

SEQ ID NO: 47 - protein, 173 aa, Artificial Sequence
  Amino acid sequence of murine TCRbeta constant region
EDLRNVTPPKVSLFEPSKAEIANKQKATLVCLARGFFPDHVELSWWVNGKEVHSGVSTDPQAYKESNYSYCLSSRLRVSATFWHNPRNHFRCQVQFHGLSEEDKWPEGSPKPVTQNISAEAWGRADCGITSASYQQGVLSATILYEILLGKATLYAVLVSTLVVMAMVKRKNS

SEQ ID NO: 48 - DNA, 519 bp, Artificial Sequence
  Nucleotide sequence of murine TCRbeta constant region
gaggacctgcgcaacgtcaccccaccaaaggtcagtttgtttgagccatcaaaggcggagatcgccaacaaacagaaagctacgctcgtgtgtttggctcggggcttcttcccagaccacgtagaactttcctggtgggtcaatggaaaggaggttcattccggagtgtccactgatccccaagcgtacaaggaatccaactatagctactgtctctcatctcggctccgggtgagtgcgacattctggcataatcctcggaaccactttcgatgccaagtgcagtttcatgggttgagcgaggaagacaagtggcccgagggcagtcctaaaccagtcactcaaaacataagcgccgaggcatggggtagagccgattgtgggattactagcgcttcataccaacaaggggtattgagcgctacaattctttacgaaattctcctcggcaaggcgacgctctacgccgtactggtgtctactctcgtggttatggcaatggtgaaacggaaaaacagc

SEQ ID NO: 49 - DNA, 819 bp, Artificial Sequence
  Nucleotide sequence of B8.2.4/TRAV+mCa
atgtcactttctagcctgctgaaggtggtcacagcttcactgtggctaggacctggcattgcccagaagataactcaaacccaaccaggaatgttcgtgcaggaaaaggaggctgtgactctggactgcacatatgacaccagtgatccaagttatggtctattctggtacaagcagcccagcagtggggaaatgatttttcttatttatcaggggtcttatgaccagcaaaatgcaacagaaggtcgctactcattgaatttccagaaggcaagaaaatccgccaaccttgtcatctccgcttcacaactgggggactcagcaatgtacttctgtgcaatgagagagaggaccggcactgccagtaaactcacctttgggactggaacaagacttcaggtcacgctcgacatccagaacccagaacctgctgtgtaccagttaaaagatcctcggtctcaggacagcaccctctgcctgttcaccgactttgactcccaaatcaatgtgccgaaaaccatggaatctggaacgttcatcactgacaaaactgtgctggacatgaaagctatggattccaagagcaatggggccattgcctggagcaaccagacaagcttcacctgccaagatatcttcaaagagaccaacgccacctaccccagttcagacgttccctgtgatgccacgttgactgagaaaagctttgaaacagatatgaacctaaactttcaaaacctgtcagttatgggactccgaatcctcctgctgaaagtagccggatttaacctgctcatgacgctgaggctgtggtccagt

SEQ ID NO: 50 - DNA, 909 bp, Artificial Sequence
  Nucleotide sequence of B8.2.4/TRBV+mCb
atgggaatcaggctcctctgtcgtgtggccttttgtttcctggctgtaggcctcgtagatgtgaaagtaacccagagctcgagatatctagtcaaaaggacgggagagaaagtttttctggaatgtgtccaggatatggaccatgaaaatatgttctggtatcgacaagacccaggtctggggctacggctgatctatttctcatatgatgttaaaatgaaagaaaaaggagatattcctgaggggtacagtgtctctagagagaagaaggagcgcttctccctgattctggagtccgccagcaccaaccagacatctatgtacctctgtgccagcagccagacggtgccgccccagcattttggtgatgggactcgactctccatcctagaggacctgcgcaacgtcaccccaccaaaggtcagtttgtttgagccatcaaaggcggagatcgccaacaaacagaaagctacgctcgtgtgtttggctcggggcttcttcccagaccacgtagaactttcctggtgggtcaatggaaaggaggttcattccggagtgtccactgatccccaagcgtacaaggaatccaactatagctactgtctctcatctcggctccgggtgagtgcgacattctggcataatcctcggaaccactttcgatgccaagtgcagtttcatgggttgagcgaggaagacaagtggcccgagggcagtcctaaaccagtcactcaaaacataagcgccgaggcatggggtagagccgattgtgggattactagcgcttcataccaacaaggggtattgagcgctacaattctttacgaaattctcctcggcaaggcgacgctctacgccgtactggtgtctactctcgtggttatggcaatggtgaaacggaaaaacagc

SEQ ID NO: 51 - protein, 188 aa, Artificial Sequence [sequence omitted]

SEQ ID NO: 52 - protein, 16 aa, Artificial Sequence
  Amino acid sequence of WT-RT6
YKLVVVGAGGVGKSAL

SEQ ID NO: 53 - DNA, 57 bp, Artificial Sequence
  Nucleotide sequence of P2A
gccaccaacttcagcctgctgaagcaggccggcgacgtggaggagaaccccggcccc

SEQ ID NO: 54 - protein, 10 aa, Artificial Sequence
  Amino acid sequence of TCR CDR3beta95Q-A
ASSATVPPQH

SEQ ID NO: 55 - protein, 10 aa, Artificial Sequence
  Amino acid sequence of TCR CDR3beta95Q-C
ASSCTVPPQH

SEQ ID NO: 56 - protein, 10 aa, Artificial Sequence
  Amino acid sequence of TCR CDR3beta95Q-D
ASSDTVPPQH

SEQ ID NO: 57 - protein, 10 aa, Artificial Sequence
  Amino acid sequence of TCR CDR3beta95Q-E
ASSETVPPQH

SEQ ID NO: 58 - protein, 10 aa, Artificial Sequence
  Amino acid sequence of TCR CDR3beta95Q-G
ASSGTVPPQH

SEQ ID NO: 59 - protein, 10 aa, Artificial Sequence
  Amino acid sequence of TCR CDR3beta95Q-H
ASSHTVPPQH

SEQ ID NO: 60 - protein, 10 aa, Artificial Sequence
  Amino acid sequence of TCR CDR3beta95Q-I
ASSITVPPQH

SEQ ID NO: 61 - protein, 10 aa, Artificial Sequence
  Amino acid sequence of TCR CDR3beta95Q-L
ASSLTVPPQH

SEQ ID NO: 62 - protein, 10 aa, Artificial Sequence
  Amino acid sequence of TCR CDR3beta95Q-M
ASSMTVPPQH

SEQ ID NO: 63 - protein, 10 aa, Artificial Sequence
  Amino acid sequence of TCR CDR3beta95Q-N
ASSNTVPPQH

SEQ ID NO: 64 - protein, 10 aa, Artificial Sequence
  Amino acid sequence of TCR CDR3beta95Q-S
ASSSTVPPQH

SEQ ID NO: 65 - protein, 10 aa, Artificial Sequence
  Amino acid sequence of TCR CDR3beta95Q-T
ASSTTVPPQH

SEQ ID NO: 66 - protein, 10 aa, Artificial Sequence
  Amino acid sequence of TCR CDR3beta95Q-V
ASSVTVPPQH

SEQ ID NO: 67 - protein, 10 aa, Artificial Sequence
  Amino acid sequence of TCR CDR3beta95Q-W
ASSWTVPPQH

SEQ ID NO: 68 - protein, 10 aa, Artificial Sequence
  Amino acid sequence of TCR CDR3beta95Q-Y
ASSYTVPPQH

SEQ ID NO: 69 - protein, 10 aa, Artificial Sequence
  Amino acid sequence of TCR CDR3beta96T-A
ASSQAVPPQH

SEQ ID NO: 70 - protein, 10 aa, Artificial Sequence
  Amino acid sequence of TCR CDR3beta96T-C
ASSQCVPPQH

SEQ ID NO: 71 - protein, 10 aa, Artificial Sequence
  Amino acid sequence of TCR CDR3beta96T-H
ASSQHVPPQH

SEQ ID NO: 72 - protein, 10 aa, Artificial Sequence
  Amino acid sequence of TCR CDR3beta96T-K
ASSQKVPPQH

SEQ ID NO: 73 - protein, 10 aa, Artificial Sequence
  Amino acid sequence of TCR CDR3beta96T-N
ASSQNVPPQH

SEQ ID NO: 74 - protein, 10 aa, Artificial Sequence
  Amino acid sequence of TCR CDR3beta96T-S
ASSQSVPPQH

SEQ ID NO: 75 - protein, 10 aa, Artificial Sequence
  Amino acid sequence of TCR CDR3beta96T-V
ASSQVVPPQH

SEQ ID NO: 76 - protein, 10 aa, Artificial Sequence
  Amino acid sequence of TCR CDR3beta96T-W
ASSQWVPPQH

SEQ ID NO: 77 - protein, 10 aa, Artificial Sequence
  Amino acid sequence of TCR CDR3beta97V-I
ASSQTIPPQH

SEQ ID NO: 78 - protein, 10 aa, Artificial Sequence
  Amino acid sequence of TCR CDR3beta97V-S
ASSQTSPPQH

SEQ ID NO: 79 - protein, 10 aa, Artificial Sequence
  Amino acid sequence of TCR CDR3beta97V-T
ASSQTTPPQH

SEQ ID NO: 80 - protein, 10 aa, Artificial Sequence
  Amino acid sequence of TCR CDR3beta98P-C
ASSQTVCPQH

SEQ ID NO: 81 - protein, 10 aa, Artificial Sequence
  Amino acid sequence of TCR CDR3beta98P-D
ASSQTVDPQH

SEQ ID NO: 82 - protein, 10 aa, Artificial Sequence
  Amino acid sequence of TCR CDR3beta98P-E
ASSQTVEPQH

SEQ ID NO: 83 - protein, 10 aa, Artificial Sequence
  Amino acid sequence of TCR CDR3beta98P-F
ASSQTVFPQH

SEQ ID NO: 84 - protein, 10 aa, Artificial Sequence
  Amino acid sequence of TCR CDR3beta98P-G
ASSQTVGPQH

SEQ ID NO: 85 - protein, 10 aa, Artificial Sequence
  Amino acid sequence of TCR CDR3beta98P-H
ASSQTVHPQH

SEQ ID NO: 86 - protein, 10 aa, Artificial Sequence
  Amino acid sequence of TCR CDR3beta98P-L
ASSQTVLPQH

SEQ ID NO: 87 - protein, 10 aa, Artificial Sequence
  Amino acid sequence of TCR CDR3beta98P-M
ASSQTVMPQH

SEQ ID NO: 88 - protein, 10 aa, Artificial Sequence
  Amino acid sequence of TCR CDR3beta98P-R
ASSQTVRPQH

SEQ ID NO: 89 - protein, 10 aa, Artificial Sequence
  Amino acid sequence of TCR CDR3beta98P-S
ASSQTVSPQH

SEQ ID NO: 90 - protein, 10 aa, Artificial Sequence
  Amino acid sequence of TCR CDR3beta98P-V
ASSQTVVPQH

SEQ ID NO: 91 - protein, 10 aa, Artificial Sequence
  Amino acid sequence of TCR CDR3beta98P-W
ASSQTVWPQH

SEQ ID NO: 92 - protein, 10 aa, Artificial Sequence
  General formula of TCR CDR3beta
  MISC_FEATURE (4)..(4): Xaa is selected from the group consisting of Gln, Ala, Cys, Asp, Glu, Gly, His, Ile, Leu, Met, Asn, Ser, Thr, Val, Trp or Tyr.
  MISC_FEATURE (5)..(5): Xaa is selected from the group consisting of Thr, Ala, Cys, His, Lys, Asn, Ser, Val or Trp.
  MISC_FEATURE (6)..(6): Xaa is selected from the group consisting of Val, Ile, Ser or Thr.
  MISC_FEATURE (7)..(7): Xaais selected from the group consisting of Pro, Cys, Asp, Glu, Phe, Gly, His, Leu, Met, Arg, Ser, Val or Trp.
ASSXXXXPQH

SEQ ID NO: 93 - protein, 46 aa, Artificial Sequence
  Amino acid sequence of FR1alpha
MSLSSLLKVVTASLWLGPGIAQKITQTQPGMFVQEKEAVTLDCTYD

SEQ ID NO: 94 - protein, 17 aa, Artificial Sequence
  Amino acid sequence of FR2alpha
LFWYKQPSSGEMIFLIY

SEQ ID NO: 95 - protein, 34 aa, Artificial Sequence
  Amino acid sequence of FR3alpha
ATEGRYSLNFQKARKSANLVISASQLGDSAMYFC

SEQ ID NO: 96 - protein, 11 aa, Artificial Sequence
  Amino acid sequence of FR4alpha
FGTGTRLQVTL

SEQ ID NO: 97 - protein, 45 aa, Artificial Sequence
  Amino acid sequence of FR1beta
MGIRLLCRVAFCFLAVGLVDVKVTQSSRYLVKRTGEKVFLECVQD

SEQ ID NO: 98 - protein, 17 aa, Artificial Sequence
  Amino acid sequence of FR2beta
MFWYRQDPGLGLRLIYF

SEQ ID NO: 99 - protein, 37 aa, Artificial Sequence
  Amino acid sequence of FR3beta
KEKGDIPEGYSVSREKKERFSLILESASTNQTSMYLC

SEQ ID NO: 100 - protein, 10 aa, Artificial Sequence
  Amino acid sequence of FR4beta
FGDGTRLSIL